European Patent Specification EP 4 071 250 B1, published March 5, 2025. Title: COMBINATORIAL DNA SCREENING. Applicant: MYRIAD WOMEN'S HEALTH, INC. Application EP. The sequence listing filed with the application follows.

SEQUENCE LISTING (12 sequences)

SEQ ID NO: 1 - DNA, 13 bp, Artificial Sequence
  Description of Artificial Sequence: Synthetic oligonucleotide
aatgccatggctt

SEQ ID NO: 2 - DNA, 13 bp, Artificial Sequence
  Description of Artificial Sequence: Synthetic oligonucleotide
cagtagctctgat

SEQ ID NO: 3 - DNA, 13 bp, Artificial Sequence
  Description of Artificial Sequence: Synthetic oligonucleotide
gacgtatacgctt

SEQ ID NO: 4 - DNA, 13 bp, Artificial Sequence
  Description of Artificial Sequence: Synthetic oligonucleotide
tacggactcgtat

SEQ ID NO: 5 - DNA, 14 bp, Artificial Sequence
  Description of Artificial Sequence: Synthetic oligonucleotide
aacgttcgagtcct

SEQ ID NO: 6 - DNA, 14 bp, Artificial Sequence
  Description of Artificial Sequence: Synthetic oligonucleotide
cacgttacgatgat

SEQ ID NO: 7 - DNA, 14 bp, Artificial Sequence
  Description of Artificial Sequence: Synthetic oligonucleotide
gctcctagacgtat

SEQ ID NO: 8 - DNA, 14 bp, Artificial Sequence
  Description of Artificial Sequence: Synthetic oligonucleotide
tatcgagctagcct

SEQ ID NO: 9 - DNA, 15 bp, Artificial Sequence
  Description of Artificial Sequence: Synthetic oligonucleotide
acgtagctgatcagt

SEQ ID NO: 10 - DNA, 15 bp, Artificial Sequence
  Description of Artificial Sequence: Synthetic oligonucleotide
caggactagcttact

SEQ ID NO: 11 - DNA, 15 bp, Artificial Sequence
  Description of Artificial Sequence: Synthetic oligonucleotide
gcatcgctagtagat

SEQ ID NO: 12 - DNA, 15 bp, Artificial Sequence
  Description of Artificial Sequence: Synthetic oligonucleotide
tacgtagtacgcagt